European Patent Application EP 4 616 705 A2, published September 17, 2025. Title: PERONOSPORA RESISTANCE IN SPINACIA OLERACEA. Applicant: Rijk Zwaan Zaadteelt en Zaadhandel B.V. Application EP. The sequence listing filed with the application follows.

SEQUENCE LISTING (14 sequences)

SEQ ID NO: 1 - DNA, 20 bp, synthetic construct
  misc_feature 1..20: note = Forward primer LRR domain (alpha)
  source 1..20: mol_type = other DNA
acaagtggatgtgtcttagg

SEQ ID NO: 2 - DNA, 19 bp, synthetic construct
  misc_feature 1..19: note = Reverse primer LRR domain (alpha)
  source 1..19: mol_type = other DNA
ttcgccctcatcttcctgg

SEQ ID NO: 3 - DNA, 18 bp, synthetic construct
  misc_feature 1..18: note = Forward primer LRR domain (beta)
  source 1..18: mol_type = other DNA
tcacgtgggttgtgttgt

SEQ ID NO: 4 - DNA, 1433 bp, Spinacia oleracea
  misc_feature 1..1433: note = Amplicon of LRR domain of the alpha-WOLF 25 allele
  source 1..1433: mol_type = genomic DNA
acaagtggatgtgtcttaggatgttggacttgtcaaattcagatgttaaaagtttgcctaattcaataggtaagttgttgcacttacggtatcttaacctgtcaaataatagaaatctaaagatacttcctgatgcaattacaagactgcataacttgcagacactacttttagaagattgcagaagtttaaaggagttgccaaaagatttttgcaaattggtcaaactgaggcacttggatttaaggttttgttctgatttgattggtatgccattgggaatggataggctaactagtcttagagtactgccattctttgtggtgggtaggaaggaacaaagtgttgatgatgagctgaaagccctaaaaggcctcaccgagataaaaggctccattcgtattagaatccattcaaagtatagaatagttgaaggcatgaatgacacaggaggagctgggtatttgaagagcatgaaacatctcacgagggttattattagatttgatgataaagaaggtggatgtgttaaccctgaagctgtgttggcaaccctagagccaccttcaaatatcaagagcttatctatagataattacgatggtacaacaattccagtatggggaagagcagagattaattgggcaatctccctctcacatcttgtcgacatccagctttggtgttgtagtaatttgcaggagatgccagtgctgagtaaactgcctcatttgaaatcactgtatctttttaagttttgtaagttagagtacatggagagtagaagcagcagcagtagcagtgacacagaagcagcaacaccagaattaccaacattcttcccttcccttgaaaaacttacactttggtatctggaaaagttgaagggttttgggaacaggagaccgagtagttttccccgcctctctaaattggaaatctgggaatgcccagatctaacgtggtttcctccttgtccaagccttaaaacgttgaaattggaaaaaaacaatgaagcgttgcaaataatagtaaaaataacaacaacaagaggtaaagaagaaaaagaagaagacaagaatgctggtgttggaaattcacaagatgatgacaatgtcaaattacggaaggtggaaatagacaatgtgagttatctcaaatcactgcccacaaattgtcttactcacctcaaaataactggaatagattacagggagggggagattgaatcagattccgtggaggaggagattgaattggaagttggggaggcatttcagaagtgtgcatcttctttgagaagcctcatcataatcggaaatcacggaataaataaagtgatgagactgtctggaagaacagggttggagcatttcactctgttggactcactcaaactttcaaatatagaagaccaggaagatgagggcgaa

SEQ ID NO: 5 - protein, 477 aa, Spinacia oleracea
  REGION 1..477: note = amino acid sequence encoded by amplicon of LRR domain of alpha-WOLF 25
KWMCLRMLDLSNSDVKSLPNSIGKLLHLRYLNLSNNRNLKILPDAITRLHNLQTLLLEDCRSLKELPKDFCKLVKLRHLDLRFCSDLIGMPLGMDRLTSLRVLPFFVVGRKEQSVDDELKALKGLTEIKGSIRIRIHSKYRIVEGMNDTGGAGYLKSMKHLTRVIIRFDDKEGGCVNPEAVLATLEPPSNIKSLSIDNYDGTTIPVWGRAEINWAISLSHLVDIQLWCCSNLQEMPVLSKLPHLKSLYLFKFCKLEYMESRSSSSSSDTEAATPELPTFFPSLEKLTLWYLEKLKGFGNRRPSSFPRLSKLEIWECPDLTWFPPCPSLKTLKLEKNNEALQIIVKITTTRGKEEKEEDKNAGVGNSQDDDNVKLRKVEIDNVSYLKSLPTNCLTHLKITGIDYREGEIESDSVEEEIELEVGEAFQKCASSLRSLIIIGNHGINKVMRLSGRTGLEHFTLLDSLKLSNIEDQEDEGE

SEQ ID NO: 6 - DNA, 1597 bp, Spinacia oleracea
  misc_feature 1..1597: note = Amplicon of LRR domain of the beta-WOLF 0 allele
  source 1..1597: mol_type = genomic DNA
tcacgtgggttgtgttgtcgatagagatccagaaatagtctttttatgtagcaataagattcgttcgtatattagcggtcgctgcataaagaatccggtggattcacaaatagacaactggatgtgccttagggtgttggacttgtcagattcatgtgttaaagatttgtctgattcaataggtaagctgctgcacttaaggtatcttaacctctcttctaatataaagttggagataatccctgatgcaattacaagactgcataacttgcagacactacttttagaagattgcagaagtttaaaggagttgccaaaagatttttgcaaattggtcaaactgaggcacttggaattacagggttgtcatgatttgattggtatgtcatttggaatggataagctaactagtcttagaatactaccaaacattgtggtgggtaggaaggaacaaagtgttgatgatgagctgaaagccctaaaaggcctcaccgagataaaaggctccattgatatcacaatctattcaaaatatagaagagttgaaggcatgaatggcacaggaggaggagctgggtatttgaagagcatgaaacatctcacgggggttaatattacatttgatgaaggtggatgtgttaaccctgaagctgtgtatttgaagagcatgaaacatctcacgagggttattattatatttgattataaaggtggatgtgttaaccctgaagctgtgttggcaaccctagagccaccttcaaatatcaagaggttagagatgtggcattacagtggtacaacaattccagtatggggaagagcagagattaattgggcaatctccctctcacatcttgtcgacatcacgcttgaagattgttacaatttgcaggagatgccagtgctgagtaaactgcctcatttgaaatcactggaacttacagagttggataacttagagtacatggagagtagaagcagcagcagtagcagtgacacagaagcagcaacaccagaattaccaacattcttcccttcccttgaaaaacttacactttggcgtctggacaagttgaagggttttgggaacaggagatcgagtagttttccccgcctctctaaattggaaatctggaaatgtccagatctaacgtcatttccttcttgtccaagccttgaagagttggaattgaaagaaaacaatgaagcgttgcaaataatagtaaaaataacaacaacaagaggtaaagaagaaaaagaagaagacaagaatgctggtgttggaaattcacaagatgatgacaatgtcaaattatggaaggtggaaatagacaatctgggttatctcaaatcactgcccacaaattgtctgactcacctcgaccttacaataagtgattccaaggagggggagggtgaatgggaagttggggatgcatttcagaagtgtgtatcttctttgagaagcctcaccataatcggaaatcacggaataaataaagtgaagagactgtctggaagaacagggttggagcatttcactctgttggaatcactcaaactttcagatatagaagaccaggaagatgagggcgaa

SEQ ID NO: 7 - protein, 532 aa, Spinacia oleracea
  REGION 1..532: note = amino acid sequence encoded by amplicon of LRR domain Beta Wolf 0 (Viroflay)
HVGCVVDRDPEIVFLCSNKIRSYISGRCIKNPVDSQIDNWMCLRVLDLSDSCVKDLSDSIGKLLHLRYLNLSSNIKLEIIPDAITRLHNLQTLLLEDCRSLKELPKDFCKLVKLRHLELQGCHDLIGMSFGMDKLTSLRILPNIVVGRKEQSVDDELKALKGLTEIKGSIDITIYSKYRRVEGMNGTGGGAGYLKSMKHLTGVNITFDEGGCVNPEAVYLKSMKHLTRVIIIFDYKGGCVNPEAVLATLEPPSNIKRLEMWHYSGTTIPVWGRAEINWAISLSHLVDITLEDCYNLQEMPVLSKLPHLKSLELTELDNLEYMESRSSSSSSDTEAATPELPTFFPSLEKLTLWRLDKLKGFGNRRSSSFPRLSKLEIWKCPDLTSFPSCPSLEELELKENNEALQIIVKITTTRGKEEKEEDKNAGVGNSQDDDNVKLWKVEIDNLGYLKSLPTNCLTHLDLTISDSKEGEGEWEVGDAFQKCVSSLRSLTIIGNHGINKVKRLSGRTGLEHFTLLESLKLSDIEDQEDEGE

SEQ ID NO: 8 - DNA, 3486 bp, Spinacia oleracea
  misc_feature 1..3486: note = coding sequence of the alpha-WOLF 25 allele
  source 1..3486: mol_type = genomic DNA
atggccgaaatcggatactcggtttgtgcgaaactcatcgaagtgattggcagtgagctgatcaaagagatttgtgacacatggggttacaaatctcttcttgaggacctcaacaaaactgtattgacggtcaggaacgttctcattcaagccggggtgatgcgggagcttactagtgaacaacaaggtttcattgcagaccttaaagatgttgtttatgatgctgatgacttgttcgacaagttactcactcgtgctgagcgaaaacagattgatggaaacgaaatctctgaaaaggtacgtcgtttcttttcctctagtaacaagatcggtcaagcttactacatgtctcgtaaggttaaggaaattaagaagcagttggatgaaattgttgataggcatacaaaatttgggtttagtgctgagtttatacctgtttgtagggaaagggggaacgagagggaaacacgttcatatatagatgtcaagaatattcttgggagggataaagataagaatgatatcattgataggttgcttaatcgtaatggtaatgaagcttgtagtttcctgaccatagtgggagcgggaggattgggaaaaactgctcttgcacaacttgtgttcaatgatgaaagggtcaaaattgagtttcatgatttgaggtattgggtttgtgtctctgatcaagatgggggccaatttgatgtgaaagaaatcctttgtaagattttagaggtggttactaaggagaaagttgataatagttccacattggaattggtgcaaagccaatttcaagagaagttaagaggaaagaagtacttccttgttctcgatgatgtatggaacgagggtcgtgagaagtggcttcatttggaagagttgttaatgttgggtcaagggggaagcaaggttgtagtgaccgcacgttcagagaagacagcaaatgtcatagggaaaagacatttttatacactggaatgtttgtcgccagattattcatggagcttatttgaaatgtcggcttttcagaaagggcatgagcaggaaaaccatgacgaactagttgatattgggaaaaagattgttgaaaaatgttataacaatccacttgctataacggtggtaggaagtcttctttatggagaggagataaataagtggcggtcatttgaaatgagtgagttggccaaaattggcaatggggataataagattttgtcgatattgaagctcagttactacaatcttgcaaactctttgaagagttgttttagttattgtgcagtatttcccaaggatcataaaatagagaaggagatgttgattgacctttggatagcacaaggatatgttgtgccgttggatggaggtcaaagtatagaagatgctgccgaggaacattttgtaattttgttacgaaggtgtttctttcaagatgtagtgaaggatgaatacggtgatgttgattctgttaaaatccacgacttgatgcacgatgtcgcccaagaagtgggcagagaggaaatctgtatagtgaatgataatacaaagaacttgggtgataaaatccgtcatgtacatcgtgatgtcattagatatgcacaaagagtctctctgtgtagccataagattcgttcgtatattggtggtaaatgtgaaaaacgttgggtggatacactaatagacaagtggatgtgtcttaggatgttggacttgtcaaattcagatgttaaaagtttgcctaattcaataggtaagttgttgcacttacggtatcttaacctgtcaaataatagaaatctaaagatacttcctgatgcaattacaagactgcataacttgcagacactacttttagaagattgcagaagtttaaaggagttgccaaaagatttttgcaaattggtcaaactgaggcacttggatttaaggttttgttctgatttgattggtatgccattgggaatggataggctaactagtcttagagtactgccattctttgtggtgggtaggaaggaacaaagtgttgatgatgagctgaaagccctaaaaggcctcaccgagataaaaggctccattcgtattagaatccattcaaagtatagaatagttgaaggcatgaatgacacaggaggagctgggtatttgaagagcatgaaacatctcacgagggttattattagatttgatgataaagaaggtggatgtgttaaccctgaagctgtgttggcaaccctagagccaccttcaaatatcaagagcttatctatagataattacgatggtacaacaattccagtatggggaagagcagagattaattgggcaatctccctctcacatcttgtcgacatccagctttggtgttgtagtaatttgcaggagatgccagtgctgagtaaactgcctcatttgaaatcactgtatctttttaagttttgtaagttagagtacatggagagtagaagcagcagcagtagcagtgacacagaagcagcaacaccagaattaccaacattcttcccttcccttgaaaaacttacactttggtatctggaaaagttgaagggttttgggaacaggagaccgagtagttttccccgcctctctaaattggaaatctgggaatgcccagatctaacgtggtttcctccttgtccaagccttaaaacgttgaaattggaaaaaaacaatgaagcgttgcaaataatagtaaaaataacaacaacaagaggtaaagaagaaaaagaagaagacaagaatgctggtgttggaaattcacaagatgatgacaatgtcaaattacggaaggtggaaatagacaatgtgagttatctcaaatcactgcccacaaattgtcttactcacctcaaaataactggaatagattacagggagggggagattgaatcagattccgtggaggaggagattgaattggaagttggggaggcatttcagaagtgtgcatcttctttgagaagcctcatcataatcggaaatcacggaataaataaagtgatgagactgtctggaagaacagggttggagcatttcactctgttggactcactcaaactttcaaatatagaagaccaggaagatgagggcgaagacaacatcatattctggaaatcctttcctcaaaacctccgcagtttggaaattgaaaactcttacaaaatgacaagtttgcccatggggatgcagtacttaacctccctccaaaccctctatctacaccatttttatgaattgaattcccttccagaatggataagcagcttatcatctcttcaatacctgcgcatatactactgtccagccctgaaatcactaccagaagcaatgcggaacctcacctcccttcagacacttgggatatcggattgtccagacctagttaaaagatgcagaaaacccaacggcaaggactatcccaaaattcaacacatccccaaaattgacatggattga

SEQ ID NO: 9 - protein, 1161 aa, Spinacia oleracea
  REGION 1..1161: note = amino acid sequence of the alpha-WOLF 25 allele
MAEIGYSVCAKLIEVIGSELIKEICDTWGYKSLLEDLNKTVLTVRNVLIQAGVMRELTSEQQGFIADLKDVVYDADDLFDKLLTRAERKQIDGNEISEKVRRFFSSSNKIGQAYYMSRKVKEIKKQLDEIVDRHTKFGFSAEFIPVCRERGNERETRSYIDVKNILGRDKDKNDIIDRLLNRNGNEACSFLTIVGAGGLGKTALAQLVFNDERVKIEFHDLRYWVCVSDQDGGQFDVKEILCKILEVVTKEKVDNSSTLELVQSQFQEKLRGKKYFLVLDDVWNEGREKWLHLEELLMLGQGGSKVVVTARSEKTANVIGKRHFYTLECLSPDYSWSLFEMSAFQKGHEQENHDELVDIGKKIVEKCYNNPLAITVVGSLLYGEEINKWRSFEMSELAKIGNGDNKILSILKLSYYNLANSLKSCFSYCAVFPKDHKIEKEMLIDLWIAQGYVVPLDGGQSIEDAAEEHFVILLRRCFFQDVVKDEYGDVDSVKIHDLMHDVAQEVGREEICIVNDNTKNLGDKIRHVHRDVIRYAQRVSLCSHKIRSYIGGKCEKRWVDTLIDKWMCLRMLDLSNSDVKSLPNSIGKLLHLRYLNLSNNRNLKILPDAITRLHNLQTLLLEDCRSLKELPKDFCKLVKLRHLDLRFCSDLIGMPLGMDRLTSLRVLPFFVVGRKEQSVDDELKALKGLTEIKGSIRIRIHSKYRIVEGMNDTGGAGYLKSMKHLTRVIIRFDDKEGGCVNPEAVLATLEPPSNIKSLSIDNYDGTTIPVWGRAEINWAISLSHLVDIQLWCCSNLQEMPVLSKLPHLKSLYLFKFCKLEYMESRSSSSSSDTEAATPELPTFFPSLEKLTLWYLEKLKGFGNRRPSSFPRLSKLEIWECPDLTWFPPCPSLKTLKLEKNNEALQIIVKITTTRGKEEKEEDKNAGVGNSQDDDNVKLRKVEIDNVSYLKSLPTNCLTHLKITGIDYREGEIESDSVEEEIELEVGEAFQKCASSLRSLIIIGNHGINKVMRLSGRTGLEHFTLLDSLKLSNIEDQEDEGEDNIIFWKSFPQNLRSLEIENSYKMTSLPMGMQYLTSLQTLYLHHFYELNSLPEWISSLSSLQYLRIYYCPALKSLPEAMRNLTSLQTLGISDCPDLVKRCRKPNGKDYPKIQHIPKIDMD

SEQ ID NO: 10 - protein, 9 aa, Spinacia oleracea
  REGION 1..9: note = N-terminal motif CC-NBS-LRR protein
MAEIGYSVC

SEQ ID NO: 11 - protein, 6 aa, Spinacia oleracea
  REGION 1..6: note = Motif CC-NBS-LRR protein
KWMCLR

SEQ ID NO: 12 - protein, 9 aa, Spinacia oleracea
  REGION 1..9: note = motif alpha-WOLF 25 allele
DQEDEGEDN

SEQ ID NO: 13 - DNA, 30 bp, synthetic construct
  misc_feature 1..30: note = Forward primer standard amplification sequence
  source 1..30: mol_type = other DNA
gcagtcgaacatgtagctgactcaggtcac

SEQ ID NO: 14 - DNA, 30 bp, synthetic construct
  misc_feature 1..30: note = Reverse primer standard amplification sequence
  source 1..30: mol_type = other DNA
tggatcacttgtgcaagcatcacatcgtag